European Patent Specification EP 3 143 148 B1, published January 3, 2024. Title: New microorganism and method for the production of 1,2-propanediol based on NADPH dependent acetol reductase and improved NADPH supply. Applicant: METABOLIC EXPLORER. The sequence listing filed with the application follows.

SEQUENCE LISTING (27 sequences)

SEQ ID NO: 1 - DNA, 101 bp, Artificial
  Oligonucleotide for frdABCD
cgtgcaaacctttcaagccgatcttgccattgtaggcgccggtggcgcgggattacgtgctgcaattgctgccgcgcaggccatatgaatatcctccttag

SEQ ID NO: 2 - DNA, 100 bp, Artificial
  Oligonucleotide for frdABCD
cgttagattgtaacgacaccaatcagcgtgacaactgtcaggatagcagccagaccgtagaaaacccatttgcccgcaggtgtaggctggagctgcttcg

SEQ ID NO: 3 - DNA, 100 bp, Artificial
  Oligonucleotide for ptsG
atgtttaagaatgcatttgctaacctgcaaaaggtcggtaaatcgctgatgctgccggtatccgtactgcctatcgcaggtgtaggctggagctgcttcg

SEQ ID NO: 4 - DNA, 100 bp, Artificial
  Oligonucleotide for ptsG
ttagtggttacggatgtactcatccatctcggttttcaggttatcggatttagtaccgaaaatcgcctgaacaccagaaccatatgaatatcctccttag

SEQ ID NO: 5 - DNA, 101 bp, Artificial
  Oligonucleotide for gldA
atggaccgcattattcaatcaccgggtaaatacatccagggcgctgatgtgattaatcgtctgggcgaatacctgaagccgtgtaggctggagctgcttcg

SEQ ID NO: 6 - DNA, 100 bp, Artificial
  Oligonucleotide for gldA
ttattcccactcttgcaggaaacgctgaccgtactggtcggctaccagcagagcggcgtaaacctgatctggcgtcgcgccatatgaatatcctccttag

SEQ ID NO: 7 - DNA, 21 bp, Artificial
  Ribosome binding site RBS120
atccggtataggaggtataga

SEQ ID NO: 8 - DNA, 261 bp, Artificial
  Sequence for recombination into pntAB
gaccgtcgaagacaattatcagtctttatccggcgttctaaggtgtttatcccactatcacggctgaatcgttaatattttgcgagttcacgccgaaatactgatttttggcgctagatcacaggcataattttcagtacgttatagggcgtttgttactaatttattttaacggagtaacatttagctcgtacatgagcagcttgtgtggctcctgacacaggcaaaccatcatcaataaaaccgatggaagggaatatc

SEQ ID NO: 9 - DNA, 260 bp, Artificial
  Sequence for recombination into pntAB
atgcgaattggcataccaagagaacggttaaccaatgaaacccgtgttgcagcaacgccaaaaacagtggaacagctgctgaaactgggttttaccgtcgcggtagagagcggcgcgggtcaactggcaagttttgacgataaagcgtttgtgcaagcgggcgctgaaattgtagaagggaatagcgtctggcagtcagagatcattctgaaggtcaatgcgccgttagatgatgaaattgcgttactgaatcctgggac

SEQ ID NO: 10 - DNA, 34 bp, Artificial
  Ribosome binding site RBS121
agacaataatcgaacaacatattaaggagagttt

SEQ ID NO: 11 - DNA, 100 bp, Artificial
  oligonucleotides for Dgpi
ccaacgcagaccgctgcctggcaggcactacagaaacacttcgatgaaatgaaagacgttacgatcgccgatctttttgctgtaggctggagctgcttcg

SEQ ID NO: 12 - DNA, 100 bp, Artificial
  oligonucleotides for Dgpi
gcgccacgctttatagcggttaatcagaccattggtcgagctatcgtggctgctgatttctttatcatctttcagctctgcatatgaatatcctccttag

SEQ ID NO: 13 - DNA, 101 bp, Artificial
  Oligonucleotide for pfkA
gttcctcggttctgcgcgtttcccggaattccgcgacgagaacatccgcgccgtggctatcgaaaacctgaaaaaacgtggtgtaggctggagctgcttcg

SEQ ID NO: 14 - DNA, 102 bp, Artificial
  Oligonucleotide for pfkA
ggcctgataagcgaagcgcatcaggcatttttgcttctgtcatcggtttcagggtaaaggaatctgcctttttccgaaatcacatatgaatatcctccttag

SEQ ID NO: 15 - DNA, 81 bp, Artificial
  oligonucleotides for recombination into Pfka
gttcctcggttctgcgcgtttcccggaattccgcgacgagaacatccgcgccgtggctatcgaaaacctgaaaaaacgtgg

SEQ ID NO: 16 - DNA, 82 bp, Artificial
  oligonucleotides for recombination into Pfka
ggcctgataagcgaagcgcatcaggcatttttgcttctgtcatcggtttcagggtaaaggaatctgcctttttccgaaatca

SEQ ID NO: 17 - DNA, 28 bp, Artificial
  Ribosome binding site RBS113
aactcatttcgtttttagggaggaataa

SEQ ID NO: 18 - DNA, 202 bp, Artificial
  Sequence for recombination into ykiA
cttccccttgaacgggagggcatttttctgaaatatcctttctttagcccataataatatttcctttgctgcgattttttcaatttccgatatattcataatttatcaaggttgatataaatatcagtgaagatctccagatattgttgcggaactggctacgataaaagataaatcagatgatgaatggtggcgtgcattg

SEQ ID NO: 19 - DNA, 254 bp, Artificial
  Sequence for recombination into ykiA
catcctgatgactggtgaactggcagcgttaattcaaaacctgattgaaggattaggtggcgaagcacaacgttaattgctgattttcctttaatgccggatgcgacgcctgccgcgtcttatccggcgtacgaagccacaccaggcatataattattcgctacggcgagcaataatttttagcgcagcaatattatgcgttttacgctgtaacttgctccatggacgttgtgtcattgtttttcctcaagccg

SEQ ID NO: 20 - DNA, 100 bp, Artificial
  Oligonucleotide for lpd
atgagtactgaaatcaaaactcaggtcgtggtacttggggcaggccccgcaggttactccgctgccttccgttgcgctgacatatgaatatcctccttag

SEQ ID NO: 21 - DNA, 100 bp, Artificial
  Oligonucleotide for lpd
ttacttcttcttcgctttcgggttcggcaggtcggtaatgctaccttcgaacacttctgccgccaggcccacagactcgttgtaggctggagctgcttcg

SEQ ID NO: 22 - DNA, 33 bp, Artificial
  Ribosome binding site RBS131
tggcaaggtaagcaaactataaggaggtcaaat

SEQ ID NO: 23 - DNA, 1013 bp, Artificial
  Synthetic gene gld
aagctttgatggcaagcgataccattcgtattccgggtattgatacaccgctgagccgtgttgcactgggcacctgggcaattggtggttggatgtggggtggtccggatgatgataatggtgttcgtaccattcatgcagcactggatgaaggtattaatctgattgataccgctccggtttatggttttggtcatagcgaagaaattgttggtcgtgcactggcagaaaaaccgaataaagcacatgttgcaaccaaactgggtctgcattgggttggtgaagatgagaaaaacatgaaagtgtttcgtgatagccgtccggcacgtattcgtaaagaagttgaagatagcctgcgtcgtctgcgtgttgaaaccattgatctggaacaaattcattggcctgatgataaaaccccgattgatgaaagcgcacgtgaactgcagaaactgcatcaggatggtaaaattcgtgccctgggtgttagcaattttagtccggaacaaatggatatctttcgtgaagttgcaccgctggcaaccattcagcctccgctgaacctgtttgaacgtaccattgaaaaagatattctgccgtatgccgaaaaacataatgcagttgttctggcatatggtgcactgtgtcgtggtctgctgaccggcaaaatgaatcgtgataccacctttccgaaagatgatctgcgtagcaatgatccgaaatttcagaaaccgaacttcgagaaatatctggctgcaatggatgagtttgaaaaactggccgagaaacgtggtaaaagcgttatggcatttgcagttcgttgggttctggatcagggtccggttattgcactgtggggtgcacgtaaaccgggtcaggttagcggtgttaaagatgtttttggttggagcctgaccgacgaagaaaaaaaagcagttgatgatattctggcacgtcatgttccgaatccgattgatccgacctttatggcaccgcctgcacgtgattaagaattc

SEQ ID NO: 24 - DNA, 971 bp, Artificial
  Synthetic gene gld2
aagctttgatggcctccaagacgtacactctgaacaccggtgccaagatacccgcggtcgggttcggcacattcgccaatgagggtgccaagggcgagacatacgcagctgttacaaaggcactggacgttggataccgccaccttgattgcgcgtggttttaccacaacgaagatgaggttggtgacgcggtacgcgattttctcgcccgccgacccgacgtgaaacgcgaggatctcttcatttgcaccaaagtttggaaccacctgcatgagccagaggacgtcaagtggagcgccaagaactcgtgcgaaaacctcaaggtcgattacattgacctgttcctcgtccactggccaatcgcggccgagaagaacagcgacaggagcgtcaagctgggccccgatggcaagtatgtcatcaaccaagccctgacggaaaacccagagccaacatggcgagccatggaagagcttgttgaaagcggcctcgtcaaggcaattggagtatccaactggacgattccggggttgaagaagctccttcagatcgccaagatcaagccggcagtgaaccagattgagattcacccattcctaccaaacgaagagcttgtggcgttctgctttgagaacgggatcctgcccgaagcctactcgccgctgggctcgcagaaccaggtcccaagcaccggcgagcgagtgcgcgacaacccgacactcaaagcggttgccgagcgaagcggctacagccttgcccagatcctattggcatggggcctgaagcgaggatatgtggtcctcccaaagagctcaactccaagccgtattgaaagcaacttcaacattccggagctgagtgatgaagactttgaggcgattcaacaggttgctaaggggagacatactagatttgtcaacatgaaggacacgtttggatacaacgtttggccagaggaggaataagaattc

SEQ ID NO: 25 - DNA, 1103 bp, Artificial
  Synthetic gene adh1
aagctttgactagtatgaaaggacttgctatgcttggaattggaagaattggatggattgaaaagaaaatcccagaatgtggaccacttgatgcattagttagaccattagcacttgcaccatgtacatcagatacacataccgtttgggcaggagctattggagatagacatgatatgattcttggacatgaagcggttggacaaattgttaaagttggatcattagttaagagattaaaagttggagataaagttattgtaccagctattacaccagattggggagaagaagaatcgcaaagaggatatccaatgcattcaggaggaatgcttggaggatggaaattctcaaatttcaaggatggagttttttcagaagttttccatgttaatgaagcagatgccaatcttgcacttcttccaagagatattaaaccagaagatgcagttatgttatcagatatggtaactactggattccatggagcagaattagctaatattaaacttggagatactgtttgtgttattggtattggaccagttggattaatgtcagttgcaggagcaaaccatcttggagcaggaagaatctttgcagtaggatcaagaaaacattgttgtgatattgcattggaatatggagcaacagatattattaattataaaaatggagatattgtagaacaaattcttaaagctacagacggcaaaggagttgataaagtcgttattgcaggaggtgatgttcatacatttgcacaagcagtcaaaatgattaaaccaggatcagatattggaaatgttaattatcttggagaaggagataatattgatattccaagaagtgaatggggagttggaatgggtcataaacacattcatggaggtttaaccccaggtggaagagtcagaatggaaaaattagcatcacttatttcaactggtaaattagatacttctaaacttattacacatagatttgaaggattagaaaaagttgaagatgcattaatgttaatgaagaataaaccagcagaccttatcaaaccagttgtcagaattcattatgatgatgaagatactcttcattaactcgag

SEQ ID NO: 26 - DNA, 101 bp, Artificial
  Oligonucleotide for yqhDE
atgaacaactttaatctgcacaccccaacccgcattctgtttggtaaaggcgcaatcgctggtttacgcgaacaaattccgtgtaggctggagctgcttcg

SEQ ID NO: 27 - DNA, 99 bp, Artificial
  Oligonucleotide for yqhDE
ttagccgccgaactggtcaggatcgggaccgagacgcttgccctgatcgagttttgcaatttcgccgagttcgtctttgcatatgaatatcctccttag